European Patent Specification EP 4 214 209 B1, published June 24, 2026. Title: RAS INHIBITORS. Applicant: Revolution Medicines, Inc. The sequence listing filed with the application follows.

SEQUENCE LISTING (4 sequences)

SEQ ID NO: 1 - DNA, 91 bp, Artificial Sequence
  Synthetic Construct
gcctgctgaaaatgactgagtataaacttgtgatggttggagcttgtggcgtaggcaagagcgccttgacgatacagctaattcagaatca

SEQ ID NO: 2 - RNA, 20 nt, Artificial Sequence
  Synthetic Construct
augguuggagcugauggcgu

SEQ ID NO: 3 - DNA, 20 bp, Artificial Sequence
  Synthetic Construct
taagtgggagcgccactcca

SEQ ID NO: 4 - DNA, 20 bp, Artificial Sequence
  Synthetic Construct
ccaaacaccagcatcaagag